European Patent Specification EP 3 491 134 B1, published October 11, 2023. Title: HUMAN INDUCED PLURIPOTENT STEM CELLS FOR HIGH EFFICIENCY GENETIC ENGINEERING. Applicant: University of Pittsburgh - Of the Commonwealth System of Higher Education Soto-Gutierrez, Alejandro Collin de l'Hortet, Alexandra  S Handa, Kan Lepe, Jorge G Takeishi, Kazuki Fox, Ira J. The sequence listing filed with the application follows.

SEQUENCE LISTING (10 sequences)

SEQ ID NO: 1 - DNA, 334 bp, Artificial Sequence
  Tetracycline inducible promoter
atcgatactagactcgagtttactccctatcagtgatagagaacgtatgaagagtttactccctatcagtgatagagaacgtatgcagactttactccctatcagtgatagagaacgtataaggagtttactccctatcagtgatagagaacgtatgaccagtttactccctatcagtgatagagaacgtatctacagtttactccctatcagtgatagagaacgtatatccagtttactccctatcagtgatagagaacgtataagctttaggcgtgtacggtgggcgcctataaaagcagagctcgtttagtgaaccgtcagatcgcctgga

SEQ ID NO: 2 - protein, 1368 aa, Streptococcus pyogenes [sequence omitted]

SEQ ID NO: 3 - DNA, 83 bp, Artificial Sequence
  tracrRNA
gttttagagctagaaatagcaagttaaaataaggctagtccgttatcaacttgaaaaagtggcaccgagtcggtgcttttttt

SEQ ID NO: 4 - DNA, 249 bp, Homo sapiens
gagggcctatttcccatgattccttcatatttgcatatacgatacaaggctgttagagagataattggaattaatttgactgtaaacacaaagatattagtacaaaatacgtgacgtagaaagtaataatttcttgggtagtttgcagttttaaaattatgttttaaaatggactatcatatgcttaccgtaacttgaaagtatttcgatttcttggctttatatatcttgtggaaaggacgaaacacc

SEQ ID NO: 5 - DNA, 378 bp, Artificial Sequence
  U6 sgRNA
ggcgcgccggatccgagggcctatttcccatgattccttcatatttgcatatacgatacaaggctgttagagagataattggaattaatttgactgtaaacacaaagatattagtacaaaatacgtgacgtagaaagtaataatttcttgggtagtttgcagttttaaaattatgttttaaaatggactatcatatgcttaccgtaacttgaaagtatttcgatttcttggctttatatatcttgtggaaaggacgaaacaccggaagagcgagctcttcggttttagagctagaaatagcaagttaaaataaggctagtccgttatcaacttgaaaaagtggcaccgagtcggtgctttttttggtaccggcgcgcc

SEQ ID NO: 6 - DNA, 966 bp, Homo sapiens
cgatacaaggctgttagagagataattagaattaatttgactgtaaacacaaagatattagtacaaaatacgtgacgtagaaagtaataatttcttgggtagtttgcagttttaaaattatgttttaaaatggactatcatatgcttaccgtaacttgaaagtatttcgatttcttggctttatatatcttgtggaaaggacgaaacaccggagacggttgtaaatgagcacacaaaatacacatgctaaaatattatattctatgacctttataaaatcaaccaaaatcttctttttaataactttagtatcaataattagaatttttatgttcctttttgcaaacttttaataaaaatgagcaaaataaaaaaacgctagttttagtaactcgcgttgttttcttcacctttaataatagctactccaccacttgttcctaagcggtcagctcctgcttcaatcattttttgagcatcttcaaatgttctaactccaccagctgctttaactaaagcattgtctttaacaactgacttcattagtttaacatcttcaaatgttgcacctgattttgaaaatcctgttgatgttttaacaaattctaatccagcttcaacagctatttcacaagctttcatgatttcttcttttgttaataaacaattttccataatacatttaacaacatgtgatccagctgctttttttacagctttcatgtcttctaaaactaattcataatttttgtcttttaatgcaccaatatttaataccatatcaatttctgttgcaccatctttaattgcttcagaaacttcgaatgcttttgtagctgttgtgcatgcacctagaggaaaacctacaacatttgttattcctacatttgtgccttttaataattctttacaatagcttgttcaatatgaattaacacaaactgttgcaaaatcaaattcaattgc

SEQ ID NO: 7 - DNA, 20 bp, Artificial Sequence
  sgRNA for EGFR promoter
tgagcttgttactcgtgcct

SEQ ID NO: 8 - DNA, 20 bp, Artificial Sequence
  sgRNA for HNF4 promoter
gggcgcgttcacgctgacca

SEQ ID NO: 9 - DNA, 21 bp, Artificial Sequence
  primer
gagggcctatttcccatgatt

SEQ ID NO: 10 - DNA, 20 bp, Artificial Sequence
  primer
gactatcatatgcttaccgt